European Patent Specification EP 4 267 763 B1, published July 23, 2025. Title: COMPOSITIONS AND METHODS FOR HIGHLY SENSITIVE DETECTION OF TARGET SEQUENCES IN MULTIPLEX REACTIONS. Applicant: Life Technologies Corporation. The sequence listing filed with the application follows.

SEQUENCE LISTING (602 sequences)

SEQ ID NO: 1 - DNA, 26 bp, Artificial Sequence
  Synthetic Sequence
tttgggctggccaaactgctgggtgc

SEQ ID NO: 2 - DNA, 25 bp, Artificial Sequence
  Synthetic Sequence
tttgggctggccaaactgctgggtg

SEQ ID NO: 3 - DNA, 24 bp, Artificial Sequence
  Synthetic Sequence
tttgggctggccaaactgctgggt

SEQ ID NO: 4 - DNA, 23 bp, Artificial Sequence
  Synthetic Sequence
tttgggctggccaaactgctggg

SEQ ID NO: 5 - DNA, 22 bp, Artificial Sequence
  Synthetic Sequence
tttgggctggccaaactgctgg

SEQ ID NO: 6 - DNA, 21 bp, Artificial Sequence
  Synthetic Sequence
tttgggctggccaaactgctg

SEQ ID NO: 7 - DNA, 20 bp, Artificial Sequence
  Synthetic Sequence
tttgggctggccaaactgct

SEQ ID NO: 8 - DNA, 19 bp, Artificial Sequence
  Synthetic Sequence
tttgggctggccaaactgc

SEQ ID NO: 9 - DNA, 18 bp, Artificial Sequence
  Synthetic Sequence
tttgggctggccaaactg

SEQ ID NO: 10 - DNA, 25 bp, Artificial Sequence
  Synthetic Sequence
ttgggctggccaaactgctgggtgc

SEQ ID NO: 11 - DNA, 24 bp, Artificial Sequence
  Synthetic Sequence
tgggctggccaaactgctgggtgc

SEQ ID NO: 12 - DNA, 23 bp, Artificial Sequence
  Synthetic Sequence
gggctggccaaactgctgggtgc

SEQ ID NO: 13 - DNA, 22 bp, Artificial Sequence
  Synthetic Sequence
ggctggccaaactgctgggtgc

SEQ ID NO: 14 - DNA, 21 bp, Artificial Sequence
  Synthetic Sequence
gctggccaaactgctgggtgc

SEQ ID NO: 15 - DNA, 20 bp, Artificial Sequence
  Synthetic Sequence
ctggccaaactgctgggtgc

SEQ ID NO: 16 - DNA, 26 bp, Artificial Sequence
  Synthetic Sequence
uuugggcuggccaaacugcugggugc

SEQ ID NO: 17 - DNA, 25 bp, Artificial Sequence
  Synthetic Sequence
uuugggcuggccaaacugcugggug

SEQ ID NO: 18 - DNA, 24 bp, Artificial Sequence
  Synthetic Sequence
uuugggcuggccaaacugcugggu

SEQ ID NO: 19 - DNA, 23 bp, Artificial Sequence
  Synthetic Sequence
uuugggcuggccaaacugcuggg

SEQ ID NO: 20 - DNA, 22 bp, Artificial Sequence
  Synthetic Sequence
uuugggcuggccaaacugcugg

SEQ ID NO: 21 - DNA, 21 bp, Artificial Sequence
  Synthetic Sequence
uuugggcuggccaaacugcug

SEQ ID NO: 22 - DNA, 20 bp, Artificial Sequence
  Synthetic Sequence
uuugggcuggccaaacugcu

SEQ ID NO: 23 - DNA, 19 bp, Artificial Sequence
  Synthetic Sequence
uuugggcuggccaaacugc

SEQ ID NO: 24 - DNA, 18 bp, Artificial Sequence
  Synthetic Sequence
uuugggcuggccaaacug

SEQ ID NO: 25 - DNA, 25 bp, Artificial Sequence
  Synthetic Sequence
uugggcuggccaaacugcugggugc

SEQ ID NO: 26 - DNA, 24 bp, Artificial Sequence
  Synthetic Sequence
ugggcuggccaaacugcugggugc

SEQ ID NO: 27 - DNA, 23 bp, Artificial Sequence
  Synthetic Sequence
gggcuggccaaacugcugggugc

SEQ ID NO: 28 - DNA, 22 bp, Artificial Sequence
  Synthetic Sequence
ggcuggccaaacugcugggugc

SEQ ID NO: 29 - DNA, 21 bp, Artificial Sequence
  Synthetic Sequence
gcuggccaaacugcugggugc

SEQ ID NO: 30 - DNA, 20 bp, Artificial Sequence
  Synthetic Sequence
cuggccaaacugcugggugc

SEQ ID NO: 31 - DNA, 18 bp, Artificial Sequence
  Synthetic Sequence
actcttcttgtccagctg

SEQ ID NO: 32 - DNA, 17 bp, Artificial Sequence
  Synthetic Sequence
aaatcactgagcaggag

SEQ ID NO: 33 - DNA, 17 bp, Artificial Sequence
  Synthetic Sequence
tgatgcacatcatggtg

SEQ ID NO: 34 - DNA, 17 bp, Artificial Sequence
  Synthetic Sequence
agccagagacatcaaga

SEQ ID NO: 35 - DNA, 17 bp, Artificial Sequence
  Synthetic Sequence
aagtgctgggctccggt

SEQ ID NO: 36 - DNA, 17 bp, Artificial Sequence
  Synthetic Sequence
gctcatcacgcagctca

SEQ ID NO: 37 - DNA, 16 bp, Artificial Sequence
  Synthetic Sequence
tttgggctggccaaac

SEQ ID NO: 38 - DNA, 18 bp, Artificial Sequence
  Synthetic Sequence
cgagatttcactgtagct

SEQ ID NO: 39 - DNA, 18 bp, Artificial Sequence
  Synthetic Sequence
ggagctggtggcgtaggc

SEQ ID NO: 40 - DNA, 24 bp, Artificial Sequence
  Synthetic Sequence
tctcatggcactgtactcttcttg

SEQ ID NO: 41 - DNA, 25 bp, Artificial Sequence
  Synthetic Sequence
tctcatggcactgtactcttcttgt

SEQ ID NO: 42 - DNA, 25 bp, Artificial Sequence
  Synthetic Sequence
ctcatggcactgtactcttcttgtc

SEQ ID NO: 43 - DNA, 24 bp, Artificial Sequence
  Synthetic Sequence
catggcactgtactcttcttgtcc

SEQ ID NO: 44 - DNA, 23 bp, Artificial Sequence
  Synthetic Sequence
tggcactgtactcttcttgtcca

SEQ ID NO: 45 - DNA, 23 bp, Artificial Sequence
  Synthetic Sequence
ccaggcacutgatgatacucact

SEQ ID NO: 46 - DNA, 24 bp, Artificial Sequence
  Synthetic Sequence
ggaagaaaaacaaucccactugcg

SEQ ID NO: 47 - DNA, 25 bp, Artificial Sequence
  Synthetic Sequence
ccattaacauggcctaccagagtug

SEQ ID NO: 48 - DNA, 23 bp, Artificial Sequence
  Synthetic Sequence
agccacacaugccatcattcuag

SEQ ID NO: 49 - DNA, 23 bp, Artificial Sequence
  Synthetic Sequence
tctggtttcuggtgggaccatua

SEQ ID NO: 50 - DNA, 28 bp, Artificial Sequence
  Synthetic Sequence
tggatcacatcuctaccagagttaauca

SEQ ID NO: 51 - DNA, 28 bp, Artificial Sequence
  Synthetic Sequence
gctattautgatggcaaauacacagagg

SEQ ID NO: 52 - DNA, 28 bp, Artificial Sequence
  Synthetic Sequence
catctacaaagtggutctggattagcug

SEQ ID NO: 53 - DNA, 21 bp, Artificial Sequence
  Synthetic Sequence
aggaggtcauggcatcgagut

SEQ ID NO: 54 - DNA, 23 bp, Artificial Sequence
  Synthetic Sequence
attaaagctggcuatggcaccug

SEQ ID NO: 55 - DNA, 18 bp, Artificial Sequence
  Synthetic Sequence
gugccaagccucacacca

SEQ ID NO: 56 - DNA, 25 bp, Artificial Sequence
  Synthetic Sequence
atttttccucacagctcgttcaucg

SEQ ID NO: 57 - DNA, 27 bp, Artificial Sequence
  Synthetic Sequence
ctttacccctccutcctagagagtuag

SEQ ID NO: 58 - DNA, 21 bp, Artificial Sequence
  Synthetic Sequence
tgcccacugtgttacugccat

SEQ ID NO: 59 - DNA, 23 bp, Artificial Sequence
  Synthetic Sequence
cattcggcacaggaugactgtua

SEQ ID NO: 60 - DNA, 29 bp, Artificial Sequence
  Synthetic Sequence
acattccgaatauagagaacctcaatcuc

SEQ ID NO: 61 - DNA, 18 bp, Artificial Sequence
  Synthetic Sequence
aggcattugccggcaguc

SEQ ID NO: 62 - DNA, 22 bp, Artificial Sequence
  Synthetic Sequence
cgccaggcucacctctatagug

SEQ ID NO: 63 - DNA, 32 bp, Artificial Sequence
  Synthetic Sequence
tgcagaaaacagauctgtatttatttcagugt

SEQ ID NO: 64 - DNA, 21 bp, Artificial Sequence
  Synthetic Sequence
cagtcctcaugtactgguccc

SEQ ID NO: 65 - DNA, 32 bp, Artificial Sequence
  Synthetic Sequence
caagatttacctcuattgttggatcatatucg

SEQ ID NO: 66 - DNA, 23 bp, Artificial Sequence
  Synthetic Sequence
cagacactguacaagctcuacga

SEQ ID NO: 67 - DNA, 23 bp, Artificial Sequence
  Synthetic Sequence
tcacagtggautcgagaagugac

SEQ ID NO: 68 - DNA, 24 bp, Artificial Sequence
  Synthetic Sequence
cattggtagcuggtgatgttccuc

SEQ ID NO: 69 - DNA, 21 bp, Artificial Sequence
  Synthetic Sequence
acacuctugagggccacaaag

SEQ ID NO: 70 - DNA, 23 bp, Artificial Sequence
  Synthetic Sequence
gctccttguagccaatgaaggug

SEQ ID NO: 71 - DNA, 20 bp, Artificial Sequence
  Synthetic Sequence
ggaccaactuggaggcctug

SEQ ID NO: 72 - DNA, 27 bp, Artificial Sequence
  Synthetic Sequence
tctattttctctuccctgcagatguca

SEQ ID NO: 73 - DNA, 19 bp, Artificial Sequence
  Synthetic Sequence
cuaggcgaggagcuccagt

SEQ ID NO: 74 - DNA, 20 bp, Artificial Sequence
  Synthetic Sequence
cattctgcuggtcgtgguct

SEQ ID NO: 75 - DNA, 28 bp, Artificial Sequence
  Synthetic Sequence
tcttctcactcauatcctcctctttcug

SEQ ID NO: 76 - DNA, 18 bp, Artificial Sequence
  Synthetic Sequence
agcguacccttgucccca

SEQ ID NO: 77 - DNA, 22 bp, Artificial Sequence
  Synthetic Sequence
gcccucccagaaggtctacaug

SEQ ID NO: 78 - DNA, 20 bp, Artificial Sequence
  Synthetic Sequence
cagctaccugaccgacgtug

SEQ ID NO: 79 - DNA, 24 bp, Artificial Sequence
  Synthetic Sequence
tcctttcgaagucatcgtcttuga

SEQ ID NO: 80 - DNA, 20 bp, Artificial Sequence
  Synthetic Sequence
ccagggucactcagctugat

SEQ ID NO: 81 - DNA, 24 bp, Artificial Sequence
  Synthetic Sequence
tctgactcagcuggtattgggaut

SEQ ID NO: 82 - DNA, 22 bp, Artificial Sequence
  Synthetic Sequence
aatgtgagcccutgagatcugc

SEQ ID NO: 83 - DNA, 18 bp, Artificial Sequence
  Synthetic Sequence
gagggcggguctcucgga

SEQ ID NO: 84 - DNA, 27 bp, Artificial Sequence
  Synthetic Sequence
acgatttccctuggagatatcgatcug

SEQ ID NO: 85 - DNA, 26 bp, Artificial Sequence
  Synthetic Sequence
atacaagtuggaaatttcugggccat

SEQ ID NO: 86 - DNA, 29 bp, Artificial Sequence
  Synthetic Sequence
aatgtcaattagcuggaacatcugaaact

SEQ ID NO: 87 - DNA, 23 bp, Artificial Sequence
  Synthetic Sequence
gacagaaaagcggcugttaguca

SEQ ID NO: 88 - DNA, 32 bp, Artificial Sequence
  Synthetic Sequence
gaatcctagtagaaugtttactaccaaaugga

SEQ ID NO: 89 - DNA, 25 bp, Artificial Sequence
  Synthetic Sequence
aaacaagacgacuttgtgacctucg

SEQ ID NO: 90 - DNA, 28 bp, Artificial Sequence
  Synthetic Sequence
tgaatggagaaacauctacaaaauccct

SEQ ID NO: 91 - DNA, 33 bp, Artificial Sequence
  Synthetic Sequence
tgtgcatatgtgtaugttgagtgtatacatuag

SEQ ID NO: 92 - DNA, 28 bp, Artificial Sequence
  Synthetic Sequence
gggaagaaaagugttttgaaatgtgtut

SEQ ID NO: 93 - DNA, 33 bp, Artificial Sequence
  Synthetic Sequence
tttattttacagaguaacagactagcuagagac

SEQ ID NO: 94 - DNA, 23 bp, Artificial Sequence
  Synthetic Sequence
gcctgctttuggagtcctatugt

SEQ ID NO: 95 - DNA, 27 bp, Artificial Sequence
  Synthetic Sequence
agttggccugaatcactatattuccat

SEQ ID NO: 96 - DNA, 30 bp, Artificial Sequence
  Synthetic Sequence
ataaatcttttctcaaugatgcttggcuct

SEQ ID NO: 97 - DNA, 17 bp, Artificial Sequence
  Synthetic Sequence
ggtggccccugagcguc

SEQ ID NO: 98 - DNA, 17 bp, Artificial Sequence
  Synthetic Sequence
gcagacutcgggcuggc

SEQ ID NO: 99 - DNA, 24 bp, Artificial Sequence
  Synthetic Sequence
ccagttacctgucctggtcattua

SEQ ID NO: 100 - DNA, 27 bp, Artificial Sequence
  Synthetic Sequence
gcacaaggaaaaautgtgaagatcugt

SEQ ID NO: 101 - DNA, 28 bp, Artificial Sequence
  Synthetic Sequence
gacatatggccauttctgttttcctgua

SEQ ID NO: 102 - DNA, 27 bp, Artificial Sequence
  Synthetic Sequence
gtgctttttgcuaaaatgcatgttucc

SEQ ID NO: 103 - DNA, 27 bp, Artificial Sequence
  Synthetic Sequence
gatctatutttccctttcuccccacag

SEQ ID NO: 104 - DNA, 33 bp, Artificial Sequence
  Synthetic Sequence
aatgaatttaaatggutttcttttctccuccaa

SEQ ID NO: 105 - DNA, 27 bp, Artificial Sequence
  Synthetic Sequence
agggcatttgcautatgaaaccaauat

SEQ ID NO: 106 - DNA, 22 bp, Artificial Sequence
  Synthetic Sequence
atggagcauctgtacagcauga

SEQ ID NO: 107 - DNA, 24 bp, Artificial Sequence
  Synthetic Sequence
ggttatgtccucattgcccucaac

SEQ ID NO: 108 - DNA, 28 bp, Artificial Sequence
  Synthetic Sequence
tcaggaaacaaaaauttgtgctaugcaa

SEQ ID NO: 109 - DNA, 19 bp, Artificial Sequence
  Synthetic Sequence
acacccaguggagaagcuc

SEQ ID NO: 110 - DNA, 27 bp, Artificial Sequence
  Synthetic Sequence
cagttaacgtctuccttctctctcugt

SEQ ID NO: 111 - DNA, 21 bp, Artificial Sequence
  Synthetic Sequence
cctccaggaagccuacgugat

SEQ ID NO: 112 - DNA, 21 bp, Artificial Sequence
  Synthetic Sequence
tgaaaacaccgcagcauguca

SEQ ID NO: 113 - DNA, 23 bp, Artificial Sequence
  Synthetic Sequence
gcttgtaagugcccgaagtguaa

SEQ ID NO: 114 - DNA, 25 bp, Artificial Sequence
  Synthetic Sequence
gcagtgcuaaccaagttctttctut

SEQ ID NO: 115 - DNA, 27 bp, Artificial Sequence
  Synthetic Sequence
aattcacagucaaggttgctgatttug

SEQ ID NO: 116 - DNA, 24 bp, Artificial Sequence
  Synthetic Sequence
ggctacaagaacuaccgauaccgt

SEQ ID NO: 117 - DNA, 26 bp, Artificial Sequence
  Synthetic Sequence
catccctgacugtgagatcaagaauc

SEQ ID NO: 118 - DNA, 25 bp, Artificial Sequence
  Synthetic Sequence
acaaaatggauccagacaactgtuc

SEQ ID NO: 119 - DNA, 33 bp, Artificial Sequence
  Synthetic Sequence
gttgttaaacataucctattatgacttgucaca

SEQ ID NO: 120 - DNA, 27 bp, Artificial Sequence
  Synthetic Sequence
acatgatagaggugacatttucaaagc

SEQ ID NO: 121 - DNA, 20 bp, Artificial Sequence
  Synthetic Sequence
ggatguacagccagtgtguc

SEQ ID NO: 122 - DNA, 25 bp, Artificial Sequence
  Synthetic Sequence
tgttgccattucagggtttcugaat

SEQ ID NO: 123 - DNA, 26 bp, Artificial Sequence
  Synthetic Sequence
ctgtgcucacacatgttctucagaat

SEQ ID NO: 124 - DNA, 20 bp, Artificial Sequence
  Synthetic Sequence
cttcttctcaucgcgggcut

SEQ ID NO: 125 - DNA, 22 bp, Artificial Sequence
  Synthetic Sequence
ttgccuagacagcaccgtaaug

SEQ ID NO: 126 - DNA, 21 bp, Artificial Sequence
  Synthetic Sequence
gggaagagccuccaccatcuc

SEQ ID NO: 127 - DNA, 24 bp, Artificial Sequence
  Synthetic Sequence
cagttcgugggcttgttttgtauc

SEQ ID NO: 128 - DNA, 28 bp, Artificial Sequence
  Synthetic Sequence
gctattautgatggcaaauacacagagg

SEQ ID NO: 129 - DNA, 28 bp, Artificial Sequence
  Synthetic Sequence
catctacaaagtggutctggattagcug

SEQ ID NO: 130 - DNA, 23 bp, Artificial Sequence
  Synthetic Sequence
attaaagctggcuatggcaccug

SEQ ID NO: 131 - DNA, 18 bp, Artificial Sequence
  Synthetic Sequence
gugccaagccucacacca

SEQ ID NO: 132 - DNA, 22 bp, Artificial Sequence
  Synthetic Sequence
tccatccugacctggtatgguc

SEQ ID NO: 133 - DNA, 25 bp, Artificial Sequence
  Synthetic Sequence
atttttccucacagctcgttcaucg

SEQ ID NO: 134 - DNA, 25 bp, Artificial Sequence
  Synthetic Sequence
cgaatgcagtutttcctcctacuca

SEQ ID NO: 135 - DNA, 23 bp, Artificial Sequence
  Synthetic Sequence
cattcggcacaggaugactgtua

SEQ ID NO: 136 - DNA, 18 bp, Artificial Sequence
  Synthetic Sequence
aggcattugccggcaguc

SEQ ID NO: 137 - DNA, 22 bp, Artificial Sequence
  Synthetic Sequence
cgccaggcucacctctatagug

SEQ ID NO: 138 - DNA, 19 bp, Artificial Sequence
  Synthetic Sequence
cggtgcgcaugtactgguc

SEQ ID NO: 139 - DNA, 33 bp, Artificial Sequence
  Synthetic Sequence
aataaaaggaattccauaacttcttgctaaguc

SEQ ID NO: 140 - DNA, 21 bp, Artificial Sequence
  Synthetic Sequence
cagtcctcaugtactgguccc

SEQ ID NO: 141 - DNA, 32 bp, Artificial Sequence; identical to SEQ ID NO: 65
  Synthetic Sequence

SEQ ID NO: 142 - DNA, 23 bp, Artificial Sequence
  Synthetic Sequence
tcacagtggautcgagaagugac

SEQ ID NO: 143 - DNA, 25 bp, Artificial Sequence
  Synthetic Sequence
ttccatagugaccaagaccatcugt

SEQ ID NO: 144 - DNA, 28 bp, Artificial Sequence
  Synthetic Sequence
auggtaagaagttguaaagagacagcct

SEQ ID NO: 145 - DNA, 21 bp, Artificial Sequence
  Synthetic Sequence
acacuctugagggccacaaag

SEQ ID NO: 146 - DNA, 20 bp, Artificial Sequence
  Synthetic Sequence
ggaccaactuggaggcctug

SEQ ID NO: 147 - DNA, 27 bp, Artificial Sequence
  Synthetic Sequence
cagctaatucatctggagaucaaaccc

SEQ ID NO: 148 - DNA, 23 bp, Artificial Sequence
  Synthetic Sequence
gggatgtttutgcagatgauggg

SEQ ID NO: 149 - DNA, 25 bp, Artificial Sequence
  Synthetic Sequence
gtatgtggcuacatgttcctgauct

SEQ ID NO: 150 - DNA, 21 bp, Artificial Sequence
  Synthetic Sequence
ctgaggaaggugaaggtgcut

SEQ ID NO: 151 - DNA, 21 bp, Artificial Sequence
  Synthetic Sequence
tgtugagggaaaacacauccc

SEQ ID NO: 152 - DNA, 18 bp, Artificial Sequence
  Synthetic Sequence
agcguacccttgucccca

SEQ ID NO: 153 - DNA, 23 bp, Artificial Sequence
  Synthetic Sequence
acaacacacagutggaggactuc

SEQ ID NO: 154 - DNA, 21 bp, Artificial Sequence
  Synthetic Sequence
gggattgcagautgggcctug

SEQ ID NO: 155 - DNA, 24 bp, Artificial Sequence
  Synthetic Sequence
tcctttcgaagucatcgtcttuga

SEQ ID NO: 156 - DNA, 20 bp, Artificial Sequence
  Synthetic Sequence
atgacctucagcagcaccuc

SEQ ID NO: 157 - DNA, 20 bp, Artificial Sequence
  Synthetic Sequence
gcagccacaccccautctug

SEQ ID NO: 158 - DNA, 18 bp, Artificial Sequence
  Synthetic Sequence
cucaccccaaugcagcga

SEQ ID NO: 159 - DNA, 25 bp, Artificial Sequence
  Synthetic Sequence
cacttcttaccutcacagccactug

SEQ ID NO: 160 - DNA, 22 bp, Artificial Sequence
  Synthetic Sequence
agggctuccatgaggaaaucca

SEQ ID NO: 161 - DNA, 26 bp, Artificial Sequence
  Synthetic Sequence
ttataaaccgtuccaaaagcaccuga

SEQ ID NO: 162 - DNA, 26 bp, Artificial Sequence
  Synthetic Sequence
caaggtgcccuattacctcaatcauc

SEQ ID NO: 163 - DNA, 23 bp, Artificial Sequence
  Synthetic Sequence
gacagaaaagcggcugttaguca

SEQ ID NO: 164 - DNA, 33 bp, Artificial Sequence
  Synthetic Sequence
aagatgaatcttctuacattttcgtaagtgtua

SEQ ID NO: 165 - DNA, 28 bp, Artificial Sequence
  Synthetic Sequence
tgaatggagaaacauctacaaaauccct

SEQ ID NO: 166 - DNA, 25 bp, Artificial Sequence
  Synthetic Sequence
gaacagguatctaccauggaggaga

SEQ ID NO: 167 - DNA, 28 bp, Artificial Sequence
  Synthetic Sequence
aaacttgtttgatuacacagacactcua

SEQ ID NO: 168 - DNA, 33 bp, Artificial Sequence; identical to SEQ ID NO: 93
  Synthetic Sequence

SEQ ID NO: 169 - DNA, 23 bp, Artificial Sequence
  Synthetic Sequence
gcctgctttuggagtcctatugt

SEQ ID NO: 170 - DNA, 27 bp, Artificial Sequence
  Synthetic Sequence
ccttagataaaacugagcaagaggcut

SEQ ID NO: 171 - DNA, 17 bp, Artificial Sequence
  Synthetic Sequence
ggtggccccugagcguc

SEQ ID NO: 172 - DNA, 18 bp, Artificial Sequence
  Synthetic Sequence
gagctgguggaggcugac

SEQ ID NO: 173 - DNA, 19 bp, Artificial Sequence
  Synthetic Sequence
caggacagccugaccucac

SEQ ID NO: 174 - DNA, 28 bp, Artificial Sequence
  Synthetic Sequence
aagctctcatguctgaactgaagauaat

SEQ ID NO: 175 - DNA, 27 bp, Artificial Sequence
  Synthetic Sequence
gcacaaggaaaaautgtgaagatcugt

SEQ ID NO: 176 - DNA, 22 bp, Artificial Sequence
  Synthetic Sequence
aatggcacggutgaatguaagg

SEQ ID NO: 177 - DNA, 24 bp, Artificial Sequence
  Synthetic Sequence
aagccctcaugtctgaacucaaag

SEQ ID NO: 178 - DNA, 29 bp, Artificial Sequence
  Synthetic Sequence
aaggttgtugaggagataaauggaaacaa

SEQ ID NO: 179 - DNA, 25 bp, Artificial Sequence
  Synthetic Sequence
tccttactcauggtcggaucacaaa

SEQ ID NO: 180 - DNA, 24 bp, Artificial Sequence
  Synthetic Sequence
ctcctaagatguccactgctgtuc

SEQ ID NO: 181 - DNA, 22 bp, Artificial Sequence
  Synthetic Sequence
atggagcauctgtacagcauga

SEQ ID NO: 182 - DNA, 20 bp, Artificial Sequence
  Synthetic Sequence
cccaccacguaccagaugga

SEQ ID NO: 183 - DNA, 21 bp, Artificial Sequence
  Synthetic Sequence
ccagtgugcccactacatuga

SEQ ID NO: 184 - DNA, 19 bp, Artificial Sequence
  Synthetic Sequence
acacccaguggagaagcuc

SEQ ID NO: 185 - DNA, 21 bp, Artificial Sequence
  Synthetic Sequence
cctccaggaagccuacgugat

SEQ ID NO: 186 - DNA, 21 bp, Artificial Sequence
  Synthetic Sequence
tgaaaacaccgcagcauguca

SEQ ID NO: 187 - DNA, 23 bp, Artificial Sequence
  Synthetic Sequence
gcttgtaagugcccgaagtguaa

SEQ ID NO: 188 - DNA, 31 bp, Artificial Sequence
  Synthetic Sequence
agaauactatagtguacacaacaaaacaggt

SEQ ID NO: 189 - DNA, 21 bp, Artificial Sequence
  Synthetic Sequence
cttctttgugggcagcatugg

SEQ ID NO: 190 - DNA, 22 bp, Artificial Sequence
  Synthetic Sequence
cctgtccuccacaggcatttut

SEQ ID NO: 191 - DNA, 25 bp, Artificial Sequence
  Synthetic Sequence
acaaaatggauccagacaactgtuc

SEQ ID NO: 192 - DNA, 33 bp, Artificial Sequence; identical to SEQ ID NO: 119
  Synthetic Sequence

SEQ ID NO: 193 - DNA, 26 bp, Artificial Sequence
  Synthetic Sequence
tccutagtctttcttugaagcagcaa

SEQ ID NO: 194 - DNA, 28 bp, Artificial Sequence
  Synthetic Sequence
acctgaaaaugacactttgtaagucaaa

SEQ ID NO: 195 - DNA, 27 bp, Artificial Sequence
  Synthetic Sequence
caaccctgtttutctccctcttatugt

SEQ ID NO: 196 - DNA, 25 bp, Artificial Sequence
  Synthetic Sequence
aacuacagaatcacaugccacacag

SEQ ID NO: 197 - DNA, 27 bp, Artificial Sequence
  Synthetic Sequence
ccaacaagattcugaagaacatgtgug

SEQ ID NO: 198 - DNA, 23 bp, Artificial Sequence
  Synthetic Sequence
ccaaaacccucctgatguacacg

SEQ ID NO: 199 - DNA, 25 bp, Artificial Sequence
  Synthetic Sequence
cccutgtggcctaugacaagaaaat

SEQ ID NO: 200 - DNA, 21 bp, Artificial Sequence
  Synthetic Sequence
ggauctcttcaugcaccggaa

SEQ ID NO: 201 - DNA, 22 bp, Artificial Sequence
  Synthetic Sequence
ctggccaagagutacgggatuc

SEQ ID NO: 202 - DNA, 28 bp, Artificial Sequence
  Synthetic Sequence
aacaagtggttauagatggtgaaaccug

SEQ ID NO: 203 - DNA, 27 bp, Artificial Sequence
  Synthetic Sequence
attaacccugattactggttuccaaca

SEQ ID NO: 204 - DNA, 25 bp, Artificial Sequence
  Synthetic Sequence
tatggtcttggacauccaggatcug

SEQ ID NO: 205 - DNA, 23 bp, Artificial Sequence
  Synthetic Sequence
gatgtgctgtugagacctctgug

SEQ ID NO: 206 - DNA, 20 bp, Artificial Sequence
  Synthetic Sequence
tgaggagaugggtggctugt

SEQ ID NO: 207 - DNA, 19 bp, Artificial Sequence
  Synthetic Sequence
cacctggcucctctucacg

SEQ ID NO: 208 - DNA, 23 bp, Artificial Sequence
  Synthetic Sequence
acttacacaucactttgcguggt

SEQ ID NO: 209 - DNA, 27 bp, Artificial Sequence
  Synthetic Sequence
tagcagccagaaaugttttgguaacag

SEQ ID NO: 210 - DNA, 21 bp, Artificial Sequence
  Synthetic Sequence
gcaatcuagcgccuggaagag

SEQ ID NO: 211 - DNA, 17 bp, Artificial Sequence
  Synthetic Sequence
gtgcgacgccutguggt

SEQ ID NO: 212 - DNA, 20 bp, Artificial Sequence
  Synthetic Sequence
gtcacugacagccctcugga

SEQ ID NO: 213 - DNA, 24 bp, Artificial Sequence
  Synthetic Sequence
tgaggagcgaugacggaatauaag

SEQ ID NO: 214 - DNA, 28 bp, Artificial Sequence
  Synthetic Sequence
ttgccutctagaacaguagacacaaaac

SEQ ID NO: 215 - DNA, 22 bp, Artificial Sequence
  Synthetic Sequence
ctgtgttuctcccttcucagga

SEQ ID NO: 216 - DNA, 27 bp, Artificial Sequence
  Synthetic Sequence
attataaggccugctgaaaatgacuga

SEQ ID NO: 217 - DNA, 25 bp, Artificial Sequence
  Synthetic Sequence
gaauaaagaggagcaggtugaggaa

SEQ ID NO: 218 - DNA, 25 bp, Artificial Sequence
  Synthetic Sequence
tagttcaacaugacgaagauggcaa

SEQ ID NO: 219 - DNA, 28 bp, Artificial Sequence
  Synthetic Sequence
agcccatttttauctacttccatctugt

SEQ ID NO: 220 - DNA, 25 bp, Artificial Sequence
  Synthetic Sequence
attgtagggtcucccttgatcugag

SEQ ID NO: 221 - DNA, 21 bp, Artificial Sequence
  Synthetic Sequence
gagggtcugacgggtagagug

SEQ ID NO: 222 - DNA, 27 bp, Artificial Sequence
  Synthetic Sequence
ctgatcttctcaaagucgtcatcctuc

SEQ ID NO: 223 - DNA, 20 bp, Artificial Sequence
  Synthetic Sequence
guaggaccttgugcccacga

SEQ ID NO: 224 - DNA, 19 bp, Artificial Sequence
  Synthetic Sequence
aacaucccacgcctagucc

SEQ ID NO: 225 - DNA, 19 bp, Artificial Sequence
  Synthetic Sequence
cgggcugggaggactucac

SEQ ID NO: 226 - DNA, 25 bp, Artificial Sequence
  Synthetic Sequence
gggcttacguctaagatttcttugt

SEQ ID NO: 227 - DNA, 20 bp, Artificial Sequence
  Synthetic Sequence
cauggtcuaagaggcagcca

SEQ ID NO: 228 - DNA, 27 bp, Artificial Sequence
  Synthetic Sequence
taattttgacatggutgggactctuga

SEQ ID NO: 229 - DNA, 24 bp, Artificial Sequence
  Synthetic Sequence
gatgatgtuctccaggucgaaagg

SEQ ID NO: 230 - DNA, 18 bp, Artificial Sequence
  Synthetic Sequence
tcucugcagggcaaacct

SEQ ID NO: 231 - DNA, 20 bp, Artificial Sequence
  Synthetic Sequence
tcctgtgtcuggccccctua

SEQ ID NO: 232 - DNA, 28 bp, Artificial Sequence
  Synthetic Sequence
gacttttcaccuctgatttctggtttut

SEQ ID NO: 233 - DNA, 18 bp, Artificial Sequence
  Synthetic Sequence
cgtggcucgggacatugc

SEQ ID NO: 234 - DNA, 23 bp, Artificial Sequence
  Synthetic Sequence
ctctctgcuctgcagcaaatuca

SEQ ID NO: 235 - DNA, 22 bp, Artificial Sequence
  Synthetic Sequence
aacaggacgaacuggattucct

SEQ ID NO: 236 - DNA, 21 bp, Artificial Sequence
  Synthetic Sequence
aataucccccggcttgugagt

SEQ ID NO: 237 - DNA, 25 bp, Artificial Sequence
  Synthetic Sequence
atgtgaacatuctgcttttcauggg

SEQ ID NO: 238 - DNA, 25 bp, Artificial Sequence
  Synthetic Sequence
tatccacatccucttcctcaggaut

SEQ ID NO: 239 - DNA, 25 bp, Artificial Sequence
  Synthetic Sequence
ttcatctugaagaagttgauggagg

SEQ ID NO: 240 - DNA, 33 bp, Artificial Sequence
  Synthetic Sequence
tgcattttagaauaggatattgtatcauaccaa

SEQ ID NO: 241 - DNA, 28 bp, Artificial Sequence
  Synthetic Sequence
aagcatcagcatutgactttaccttauc

SEQ ID NO: 242 - DNA, 25 bp, Artificial Sequence
  Synthetic Sequence
ggattggaacaagguactcttugag

SEQ ID NO: 243 - DNA, 30 bp, Artificial Sequence
  Synthetic Sequence
tttccagatacuagagtgtctgtgtaauca

SEQ ID NO: 244 - DNA, 32 bp, Artificial Sequence
  Synthetic Sequence
aagaaaaagaaacagagaauctccatttuagc

SEQ ID NO: 245 - DNA, 26 bp, Artificial Sequence
  Synthetic Sequence
tgcagugaaaagagtcucaaacacaa

SEQ ID NO: 246 - DNA, 27 bp, Artificial Sequence
  Synthetic Sequence
tgacgatcuccaattcccaaaaugaag

SEQ ID NO: 247 - DNA, 26 bp, Artificial Sequence
  Synthetic Sequence
tcatgaaatacuccaaagcctctugc

SEQ ID NO: 248 - DNA, 18 bp, Artificial Sequence
  Synthetic Sequence
gggctgugcgtcactgua

SEQ ID NO: 249 - DNA, 18 bp, Artificial Sequence
  Synthetic Sequence
ggagggugugggaaggcg

SEQ ID NO: 250 - DNA, 26 bp, Artificial Sequence
  Synthetic Sequence
ggaaactcccaucttgagtcauaagg

SEQ ID NO: 251 - DNA, 28 bp, Artificial Sequence
  Synthetic Sequence
ttagagattaaagugaaggaggaugagc

SEQ ID NO: 252 - DNA, 28 bp, Artificial Sequence
  Synthetic Sequence
ctcagttccuggacaaaaataccaauct

SEQ ID NO: 253 - DNA, 25 bp, Artificial Sequence
  Synthetic Sequence
gcaggctccaaguagattcacaaua

SEQ ID NO: 254 - DNA, 28 bp, Artificial Sequence
  Synthetic Sequence
ggaaactcccauttgtgatcauaaggaa

SEQ ID NO: 255 - DNA, 27 bp, Artificial Sequence
  Synthetic Sequence
atcattcttgaugtctctggcuagacc

SEQ ID NO: 256 - DNA, 25 bp, Artificial Sequence
  Synthetic Sequence
ttgtctgctgaaugaaccccaauac

SEQ ID NO: 257 - DNA, 20 bp, Artificial Sequence
  Synthetic Sequence
aagtggcttuggtccgtcuc

SEQ ID NO: 258 - DNA, 32 bp, Artificial Sequence
  Synthetic Sequence
atttgcatcatagutagataagactgcuaagg

SEQ ID NO: 259 - DNA, 22 bp, Artificial Sequence
  Synthetic Sequence
cagaaagcggugacttacugca

SEQ ID NO: 260 - DNA, 19 bp, Artificial Sequence
  Synthetic Sequence
tgugccagggacctuacct

SEQ ID NO: 261 - DNA, 25 bp, Artificial Sequence
  Synthetic Sequence
ctcacatcgaggauttccttgtugg

SEQ ID NO: 262 - DNA, 21 bp, Artificial Sequence
  Synthetic Sequence
gtgtucccggacataguccag

SEQ ID NO: 263 - DNA, 24 bp, Artificial Sequence
  Synthetic Sequence
caggaaaatgcuggctgaccuaaa

SEQ ID NO: 264 - DNA, 27 bp, Artificial Sequence
  Synthetic Sequence
cacaacccacugaggtatatgtauagg

SEQ ID NO: 265 - DNA, 27 bp, Artificial Sequence
  Synthetic Sequence
aaaatgccactuactgttcaaggatut

SEQ ID NO: 266 - DNA, 24 bp, Artificial Sequence
  Synthetic Sequence
aguttgcagacttuccaaagccat

SEQ ID NO: 267 - DNA, 22 bp, Artificial Sequence
  Synthetic Sequence
attttgtugcccaactggucct

SEQ ID NO: 268 - DNA, 20 bp, Artificial Sequence
  Synthetic Sequence
accagguacgcctccagaug

SEQ ID NO: 269 - DNA, 33 bp, Artificial Sequence
  Synthetic Sequence
gttttcctttacttacuacacctcagatataut

SEQ ID NO: 270 - DNA, 24 bp, Artificial Sequence
  Synthetic Sequence
gggagattccugatgggcagatua

SEQ ID NO: 271 - DNA, 33 bp, Artificial Sequence
  Synthetic Sequence
aagtttgtaagtagugctatatttatgtugact

SEQ ID NO: 272 - DNA, 20 bp, Artificial Sequence
  Synthetic Sequence
gggcattcccugcacttcua

SEQ ID NO: 273 - DNA, 27 bp, Artificial Sequence
  Synthetic Sequence
ttccttcuaaaaggccatgaagatcug

SEQ ID NO: 274 - DNA, 30 bp, Artificial Sequence
  Synthetic Sequence
aacccacatttccuttatagatgtttctuc

SEQ ID NO: 275 - DNA, 21 bp, Artificial Sequence
  Synthetic Sequence
ctgttggucacagctccagug

SEQ ID NO: 276 - DNA, 26 bp, Artificial Sequence
  Synthetic Sequence
aggataaagaccuggtccauggaaat

SEQ ID NO: 277 - DNA, 21 bp, Artificial Sequence
  Synthetic Sequence
agacaggucucccacaaacac

SEQ ID NO: 278 - DNA, 28 bp, Artificial Sequence
  Synthetic Sequence
atatattcccgttuttagggagcagaut

SEQ ID NO: 279 - DNA, 28 bp, Artificial Sequence
  Synthetic Sequence
aacaagtggttauagatggtgaaaccug

SEQ ID NO: 280 - DNA, 27 bp, Artificial Sequence
  Synthetic Sequence
attaacccugattactggttuccaaca

SEQ ID NO: 281 - DNA, 23 bp, Artificial Sequence
  Synthetic Sequence
gatgtgctgtugagacctctgug

SEQ ID NO: 282 - DNA, 20 bp, Artificial Sequence
  Synthetic Sequence
tgaggagaugggtggctugt

SEQ ID NO: 283 - DNA, 22 bp, Artificial Sequence
  Synthetic Sequence
ctgctucaggacgttgaacuct

SEQ ID NO: 284 - DNA, 19 bp, Artificial Sequence
  Synthetic Sequence
cacctggcucctctucacg

SEQ ID NO: 285 - DNA, 26 bp, Artificial Sequence
  Synthetic Sequence
agaaagaccttuctgatctggtguca

SEQ ID NO: 286 - DNA, 21 bp, Artificial Sequence
  Synthetic Sequence
gcaatcuagcgccuggaagag

SEQ ID NO: 287 - DNA, 20 bp, Artificial Sequence
  Synthetic Sequence
gtcacugacagccctcugga

SEQ ID NO: 288 - DNA, 24 bp, Artificial Sequence
  Synthetic Sequence
tgaggagcgaugacggaatauaag

SEQ ID NO: 289 - DNA, 22 bp, Artificial Sequence
  Synthetic Sequence
tgtcctccugcaggattccuac

SEQ ID NO: 290 - DNA, 31 bp, Artificial Sequence
  Synthetic Sequence
ccagagaacaaatuaaaagagttaaggacuc

SEQ ID NO: 291 - DNA, 22 bp, Artificial Sequence
  Synthetic Sequence
ctgtgttuctcccttcucagga

SEQ ID NO: 292 - DNA, 27 bp, Artificial Sequence
  Synthetic Sequence
attataaggccugctgaaaatgacuga

SEQ ID NO: 293 - DNA, 25 bp, Artificial Sequence
  Synthetic Sequence
tagttcaacaugacgaagauggcaa

SEQ ID NO: 294 - DNA, 26 bp, Artificial Sequence
  Synthetic Sequence
aaagggtacauacaaagcagtctgug

SEQ ID NO: 295 - DNA, 22 bp, Artificial Sequence
  Synthetic Sequence
catcaatgtugctcgaguccac

SEQ ID NO: 296 - DNA, 25 bp, Artificial Sequence
  Synthetic Sequence
attgtagggtcucccttgatcugag

SEQ ID NO: 297 - DNA, 27 bp, Artificial Sequence
  Synthetic Sequence
ctgatcttctcaaagucgtcatcctuc

SEQ ID NO: 298 - DNA, 22 bp, Artificial Sequence
  Synthetic Sequence
agatactgauctcgccaucgct

SEQ ID NO: 299 - DNA, 23 bp, Artificial Sequence
  Synthetic Sequence
gctgcagugggaccactattauc

SEQ ID NO: 300 - DNA, 21 bp, Artificial Sequence
  Synthetic Sequence
cacttcucacaccgctgtgut

SEQ ID NO: 301 - DNA, 20 bp, Artificial Sequence
  Synthetic Sequence
cttgccccucccaucagaac

SEQ ID NO: 302 - DNA, 21 bp, Artificial Sequence
  Synthetic Sequence
cuccccaaaccccaaugaaga

SEQ ID NO: 303 - DNA, 20 bp, Artificial Sequence
  Synthetic Sequence
cauggtcuaagaggcagcca

SEQ ID NO: 304 - DNA, 25 bp, Artificial Sequence
  Synthetic Sequence
catcacacaccauaacuccacacat

SEQ ID NO: 305 - DNA, 26 bp, Artificial Sequence
  Synthetic Sequence
aacatgatggaugtcacgttcucaaa

SEQ ID NO: 306 - DNA, 18 bp, Artificial Sequence
  Synthetic Sequence
tcucugcagggcaaacct

SEQ ID NO: 307 - DNA, 19 bp, Artificial Sequence
  Synthetic Sequence
ctcacuggcctcttcugct

SEQ ID NO: 308 - DNA, 21 bp, Artificial Sequence
  Synthetic Sequence
cccuggaagaguggccaagat

SEQ ID NO: 309 - DNA, 27 bp, Artificial Sequence
  Synthetic Sequence
gctgctgaaaaugtaactttgtaucct

SEQ ID NO: 310 - DNA, 26 bp, Artificial Sequence
  Synthetic Sequence
ttgactctgtcucctcttgtcttcuc

SEQ ID NO: 311 - DNA, 21 bp, Artificial Sequence
  Synthetic Sequence
cggactctguaggctgcagut

SEQ ID NO: 312 - DNA, 24 bp, Artificial Sequence
  Synthetic Sequence
tgcagttgguggaaccattaacuc

SEQ ID NO: 313 - DNA, 24 bp, Artificial Sequence
  Synthetic Sequence
ctttaacaccuccagtccctcauc

SEQ ID NO: 314 - DNA, 25 bp, Artificial Sequence
  Synthetic Sequence
tatccacatccucttcctcaggaut

SEQ ID NO: 315 - DNA, 27 bp, Artificial Sequence
  Synthetic Sequence
cggttgcctacuggttcaattacttut

SEQ ID NO: 316 - DNA, 28 bp, Artificial Sequence
  Synthetic Sequence
aagcatcagcatutgactttaccttauc

SEQ ID NO: 317 - DNA, 33 bp, Artificial Sequence
  Synthetic Sequence
actgctaaacactaauataacctttggaaauat

SEQ ID NO: 318 - DNA, 29 bp, Artificial Sequence
  Synthetic Sequence
actttatttggauttgatccaguaacacc

SEQ ID NO: 319 - DNA, 32 bp, Artificial Sequence; identical to SEQ ID NO: 244
  Synthetic Sequence

SEQ ID NO: 320 - DNA, 26 bp, Artificial Sequence
  Synthetic Sequence
tgcagugaaaagagtcucaaacacaa

SEQ ID NO: 321 - DNA, 28 bp, Artificial Sequence
  Synthetic Sequence
agttcaatgcaugctgtttaattgtgug

SEQ ID NO: 322 - DNA, 18 bp, Artificial Sequence
  Synthetic Sequence
gggctgugcgtcactgua

SEQ ID NO: 323 - DNA, 19 bp, Artificial Sequence
  Synthetic Sequence
gagcccaggccuttctugg

SEQ ID NO: 324 - DNA, 17 bp, Artificial Sequence
  Synthetic Sequence
catgcgguggcccucct

SEQ ID NO: 325 - DNA, 25 bp, Artificial Sequence
  Synthetic Sequence
acaaccacaugtgtccagugaaaat

SEQ ID NO: 326 - DNA, 28 bp, Artificial Sequence
  Synthetic Sequence
ttagagattaaagugaaggaggaugagc

SEQ ID NO: 327 - DNA, 27 bp, Artificial Sequence
  Synthetic Sequence
gatatgguagacagagcctaaacaucc

SEQ ID NO: 328 - DNA, 30 bp, Artificial Sequence
  Synthetic Sequence
tgttttgataaccugacagacaauaaaagg

SEQ ID NO: 329 - DNA, 24 bp, Artificial Sequence
  Synthetic Sequence
acatggaaagccccugtttcauac

SEQ ID NO: 330 - DNA, 21 bp, Artificial Sequence
  Synthetic Sequence
cttugcaggactgucaagcag

SEQ ID NO: 331 - DNA, 27 bp, Artificial Sequence
  Synthetic Sequence
autttacagtactctuccaacccaaga

SEQ ID NO: 332 - DNA, 20 bp, Artificial Sequence
  Synthetic Sequence
aagtggcttuggtccgtcuc

SEQ ID NO: 333 - DNA, 20 bp, Artificial Sequence
  Synthetic Sequence
gcgggacaaggaugccugac

SEQ ID NO: 334 - DNA, 21 bp, Artificial Sequence
  Synthetic Sequence
cgtaggugcagtttggauggc

SEQ ID NO: 335 - DNA, 19 bp, Artificial Sequence
  Synthetic Sequence
tgugccagggacctuacct

SEQ ID NO: 336 - DNA, 21 bp, Artificial Sequence
  Synthetic Sequence
gtgtucccggacataguccag

SEQ ID NO: 337 - DNA, 24 bp, Artificial Sequence
  Synthetic Sequence
caggaaaatgcuggctgaccuaaa

SEQ ID NO: 338 - DNA, 27 bp, Artificial Sequence
  Synthetic Sequence
cacaacccacugaggtatatgtauagg

SEQ ID NO: 339 - DNA, 32 bp, Artificial Sequence
  Synthetic Sequence
taaaagaggagaaacucagagataaccaauac

SEQ ID NO: 340 - DNA, 21 bp, Artificial Sequence
  Synthetic Sequence
tccctgtaccutcacctcugg

SEQ ID NO: 341 - DNA, 21 bp, Artificial Sequence
  Synthetic Sequence
tcacagcacauagucccggaa

SEQ ID NO: 342 - DNA, 33 bp, Artificial Sequence; identical to SEQ ID NO: 269
  Synthetic Sequence

SEQ ID NO: 343 - DNA, 24 bp, Artificial Sequence
  Synthetic Sequence
gggagattccugatgggcagatua

SEQ ID NO: 344 - DNA, 27 bp, Artificial Sequence
  Synthetic Sequence
cagatgctcugagaaaggcatuagaaa

SEQ ID NO: 345 - DNA, 28 bp, Artificial Sequence
  Synthetic Sequence
ctcctctagcuatcttaatgactuggac

SEQ ID NO: 346 - DNA, 24 bp, Artificial Sequence
  Synthetic Sequence
atctcugccatcattuccggaaag

SEQ ID NO: 347 - DNA, 16 bp, Artificial Sequence
  Synthetic Sequence
cagcctccagttcagc

SEQ ID NO: 348 - DNA, 17 bp, Artificial Sequence
  Synthetic Sequence
cacagcaacaccctggt

SEQ ID NO: 349 - DNA, 17 bp, Artificial Sequence
  Synthetic Sequence
cgtccagggcttcttcc

SEQ ID NO: 350 - DNA, 14 bp, Artificial Sequence
  Synthetic Sequence
gcctcgaggcagcg

SEQ ID NO: 351 - DNA, 20 bp, Artificial Sequence
  Synthetic Sequence
tctcaccaagtagctcaggg

SEQ ID NO: 352 - DNA, 21 bp, Artificial Sequence
  Synthetic Sequence
ccattcattgaaacctcagcc

SEQ ID NO: 353 - DNA, 24 bp, Artificial Sequence
  Synthetic Sequence
catactggatacagctggacaaga

SEQ ID NO: 354 - DNA, 19 bp, Artificial Sequence
  Synthetic Sequence
tgcgcttttcccaacacca

SEQ ID NO: 355 - DNA, 27 bp, Artificial Sequence
  Synthetic Sequence
ccatgtacaagatcaattacagtcggg

SEQ ID NO: 356 - DNA, 19 bp, Artificial Sequence
  Synthetic Sequence
ggaggagaagtgcttctgc

SEQ ID NO: 357 - DNA, 17 bp, Artificial Sequence
  Synthetic Sequence
ccactgtgcgacgagct

SEQ ID NO: 358 - DNA, 20 bp, Artificial Sequence
  Synthetic Sequence
ccagaaacatcctggtagct

SEQ ID NO: 359 - DNA, 20 bp, Artificial Sequence
  Synthetic Sequence
gggattcaattgccatccat

SEQ ID NO: 360 - DNA, 24 bp, Artificial Sequence
  Synthetic Sequence
ccatcgacttacattggtggtctt

SEQ ID NO: 361 - DNA, 26 bp, Artificial Sequence
  Synthetic Sequence
gcgattaagaagacccctatgcagta

SEQ ID NO: 362 - DNA, 14 bp, Artificial Sequence
  Synthetic Sequence
accggcggcctaga

SEQ ID NO: 363 - DNA, 16 bp, Artificial Sequence
  Synthetic Sequence
ggccggtgaggcgatc

SEQ ID NO: 364 - DNA, 13 bp, Artificial Sequence
  Synthetic Sequence
cgccggcggtgtg

SEQ ID NO: 365 - DNA, 21 bp, Artificial Sequence
  Synthetic Sequence
cctgtcttgtctttgctgatg

SEQ ID NO: 366 - DNA, 20 bp, Artificial Sequence
  Synthetic Sequence
cactgtactcctcttgacct

SEQ ID NO: 367 - DNA, 18 bp, Artificial Sequence
  Synthetic Sequence
tagttggagctggtggcg

SEQ ID NO: 368 - DNA, 18 bp, Artificial Sequence
  Synthetic Sequence
tgaggtggtgatggggaa

SEQ ID NO: 369 - DNA, 19 bp, Artificial Sequence
  Synthetic Sequence
tcctcgtggccatgaatga

SEQ ID NO: 370 - DNA, 23 bp, Artificial Sequence
  Synthetic Sequence
tgacacaggatgtttgatccacc

SEQ ID NO: 371 - DNA, 19 bp, Artificial Sequence
  Synthetic Sequence
cgcacgtctgtaggggagt

SEQ ID NO: 372 - DNA, 20 bp, Artificial Sequence
  Synthetic Sequence
cttctgggtaagaaaggcct

SEQ ID NO: 373 - DNA, 19 bp, Artificial Sequence
  Synthetic Sequence
tcaactcccgtggggagat

SEQ ID NO: 374 - DNA, 19 bp, Artificial Sequence
  Synthetic Sequence
cccatcaccattggcaggc

SEQ ID NO: 375 - DNA, 16 bp, Artificial Sequence
  Synthetic Sequence
ctcatcaagcgacggc

SEQ ID NO: 376 - DNA, 21 bp, Artificial Sequence
  Synthetic Sequence
gggatgtgttttccctcaaca

SEQ ID NO: 377 - DNA, 19 bp, Artificial Sequence
  Synthetic Sequence
gccaagtccctgtgtacga

SEQ ID NO: 378 - DNA, 14 bp, Artificial Sequence
  Synthetic Sequence
ggtgggcacgcgga

SEQ ID NO: 379 - DNA, 19 bp, Artificial Sequence
  Synthetic Sequence
ccttggctttctgggtgag

SEQ ID NO: 380 - DNA, 14 bp, Artificial Sequence
  Synthetic Sequence
gccccctcccgagc

SEQ ID NO: 381 - DNA, 19 bp, Artificial Sequence
  Synthetic Sequence
gatgatgtgggtgggctgt

SEQ ID NO: 382 - DNA, 19 bp, Artificial Sequence
  Synthetic Sequence
aaaccacttcatccaccgg

SEQ ID NO: 383 - DNA, 17 bp, Artificial Sequence
  Synthetic Sequence
ccgccatgagctccagc

SEQ ID NO: 384 - DNA, 18 bp, Artificial Sequence
  Synthetic Sequence
tggaagccctgatcatca

SEQ ID NO: 385 - DNA, 23 bp, Artificial Sequence
  Synthetic Sequence
ctatcatcataggtcgtcatgct

SEQ ID NO: 386 - DNA, 19 bp, Artificial Sequence
  Synthetic Sequence
ctggcaattgtgacccagt

SEQ ID NO: 387 - DNA, 20 bp, Artificial Sequence
  Synthetic Sequence
agcaacagtcttacctggac

SEQ ID NO: 388 - DNA, 20 bp, Artificial Sequence
  Synthetic Sequence
gtgactttagaatgcctccg

SEQ ID NO: 389 - DNA, 20 bp, Artificial Sequence
  Synthetic Sequence
cataagggttctcctccatg

SEQ ID NO: 390 - DNA, 19 bp, Artificial Sequence
  Synthetic Sequence
ccatgccaatggacagtgt

SEQ ID NO: 391 - DNA, 21 bp, Artificial Sequence
  Synthetic Sequence
ggatgtatttgaagcacctga

SEQ ID NO: 392 - DNA, 22 bp, Artificial Sequence
  Synthetic Sequence
ctacacagtatccagcacatga

SEQ ID NO: 393 - DNA, 24 bp, Artificial Sequence
  Synthetic Sequence
cagttttatctaaggctagggtct

SEQ ID NO: 394 - DNA, 17 bp, Artificial Sequence
  Synthetic Sequence
ccccacagagcgctccc

SEQ ID NO: 395 - DNA, 20 bp, Artificial Sequence
  Synthetic Sequence
tgaaattcgctggagggtca

SEQ ID NO: 396 - DNA, 16 bp, Artificial Sequence
  Synthetic Sequence
ggcctggccagagaca

SEQ ID NO: 397 - DNA, 22 bp, Artificial Sequence
  Synthetic Sequence
ccagaaatcctgacttacgaca

SEQ ID NO: 398 - DNA, 22 bp, Artificial Sequence
  Synthetic Sequence
caaggtaactcaggactttgag

SEQ ID NO: 399 - DNA, 22 bp, Artificial Sequence
  Synthetic Sequence
cccatgtatgaagtacagtgga

SEQ ID NO: 400 - DNA, 18 bp, Artificial Sequence
  Synthetic Sequence
agacttggcagccagaaa

SEQ ID NO: 401 - DNA, 20 bp, Artificial Sequence
  Synthetic Sequence
tggaactgatggagggagga

SEQ ID NO: 402 - DNA, 16 bp, Artificial Sequence
  Synthetic Sequence
cgtggtgcccctctat

SEQ ID NO: 403 - DNA, 28 bp, Artificial Sequence
  Synthetic Sequence
gaattttcgtagtacatatttcctctga

SEQ ID NO: 404 - DNA, 23 bp, Artificial Sequence
  Synthetic Sequence
agctgttttcacctctgttgctt

SEQ ID NO: 405 - DNA, 24 bp, Artificial Sequence
  Synthetic Sequence
tcttgaggatcttgaaggaaactg

SEQ ID NO: 406 - DNA, 26 bp, Artificial Sequence
  Synthetic Sequence
gagatgttgcttctcttaattccttg

SEQ ID NO: 407 - DNA, 15 bp, Artificial Sequence
  Synthetic Sequence
tgatggccagcgtgg

SEQ ID NO: 408 - DNA, 20 bp, Artificial Sequence
  Synthetic Sequence
acagattttgggctggccaa

SEQ ID NO: 409 - DNA, 24 bp, Artificial Sequence
  Synthetic Sequence
ggcattttggttgtgtatatcatg

SEQ ID NO: 410 - DNA, 21 bp, Artificial Sequence
  Synthetic Sequence
tcttgccagagacatgtatga

SEQ ID NO: 411 - DNA, 17 bp, Artificial Sequence
  Synthetic Sequence
cccaatcggcctggtgc

SEQ ID NO: 412 - DNA, 18 bp, Artificial Sequence
  Synthetic Sequence
gccttggtccagacccag

SEQ ID NO: 413 - DNA, 22 bp, Artificial Sequence
  Synthetic Sequence
ccactccatcgagatttcactg

SEQ ID NO: 414 - DNA, 30 bp, Artificial Sequence
  Synthetic Sequence
ggacaaagaattggatctggatcatttgga

SEQ ID NO: 415 - DNA, 23 bp, Artificial Sequence
  Synthetic Sequence
attttcttctctctgacctttgg

SEQ ID NO: 416 - DNA, 24 bp, Artificial Sequence
  Synthetic Sequence
ctaggcacttactaatgctgaaga

SEQ ID NO: 417 - DNA, 22 bp, Artificial Sequence
  Synthetic Sequence
tgaggtttttccgaagagatgt

SEQ ID NO: 418 - DNA, 20 bp, Artificial Sequence
  Synthetic Sequence
ccctcatctacccactgaca

SEQ ID NO: 419 - DNA, 24 bp, Artificial Sequence
  Synthetic Sequence
tgtagtgtagcacagcttcgaagt

SEQ ID NO: 420 - DNA, 16 bp, Artificial Sequence
  Synthetic Sequence
ctcctcctggcccgtg

SEQ ID NO: 421 - DNA, 22 bp, Artificial Sequence
  Synthetic Sequence
gtacctctatggcgtctgtgtc

SEQ ID NO: 422 - DNA, 24 bp, Artificial Sequence
  Synthetic Sequence
ccttgttggcaaatcacacttgtt

SEQ ID NO: 423 - DNA, 22 bp, Artificial Sequence
  Synthetic Sequence
tgttggacatactggatacagc

SEQ ID NO: 424 - DNA, 20 bp, Artificial Sequence
  Synthetic Sequence
cttttcccaacaccacctgc

SEQ ID NO: 425 - DNA, 18 bp, Artificial Sequence
  Synthetic Sequence
cctgaggaggagaagtgc

SEQ ID NO: 426 - DNA, 14 bp, Artificial Sequence
  Synthetic Sequence
cgagctgtgccgca

SEQ ID NO: 427 - DNA, 28 bp, Artificial Sequence
  Synthetic Sequence
cctcttcacgtaggaatcctcttcataa

SEQ ID NO: 428 - DNA, 20 bp, Artificial Sequence
  Synthetic Sequence
tgcaggctccaagaagattt

SEQ ID NO: 429 - DNA, 23 bp, Artificial Sequence
  Synthetic Sequence
agattacagcttccccagactac

SEQ ID NO: 430 - DNA, 14 bp, Artificial Sequence
  Synthetic Sequence
gggccggtgaggcg

SEQ ID NO: 431 - DNA, 12 bp, Artificial Sequence
  Synthetic Sequence
gtgggcgccggc

SEQ ID NO: 432 - DNA, 19 bp, Artificial Sequence
  Synthetic Sequence
tggcgctgtactcctcctg

SEQ ID NO: 433 - DNA, 31 bp, Artificial Sequence
  Synthetic Sequence
atgtacctatggtcctagtaggaaataaatg

SEQ ID NO: 434 - DNA, 23 bp, Artificial Sequence
  Synthetic Sequence
ctgtactcctcttgacctgctgt

SEQ ID NO: 435 - DNA, 18 bp, Artificial Sequence
  Synthetic Sequence
tggtagttggagctggtg

SEQ ID NO: 436 - DNA, 14 bp, Artificial Sequence
  Synthetic Sequence
ccctcgcaccacgc

SEQ ID NO: 437 - DNA, 14 bp, Artificial Sequence
  Synthetic Sequence
gcagcccccggcac

SEQ ID NO: 438 - DNA, 18 bp, Artificial Sequence
  Synthetic Sequence
agcctgttccctcacagg

SEQ ID NO: 439 - DNA, 21 bp, Artificial Sequence
  Synthetic Sequence
cagttctcccaccttctgctt

SEQ ID NO: 440 - DNA, 19 bp, Artificial Sequence
  Synthetic Sequence
gcccacgatgtacggagag

SEQ ID NO: 441 - DNA, 19 bp, Artificial Sequence
  Synthetic Sequence
ccccaggatgttccggata

SEQ ID NO: 442 - DNA, 16 bp, Artificial Sequence
  Synthetic Sequence
ggacgtgggatcctgc

SEQ ID NO: 443 - DNA, 17 bp, Artificial Sequence
  Synthetic Sequence
ggcgcttttggcacagt

SEQ ID NO: 444 - DNA, 26 bp, Artificial Sequence
  Synthetic Sequence
cccaaagccaacaaagaaatcttaga

SEQ ID NO: 445 - DNA, 20 bp, Artificial Sequence
  Synthetic Sequence
ggtgtgggctccccatatgt

SEQ ID NO: 446 - DNA, 14 bp, Artificial Sequence
  Synthetic Sequence
ccgccggcggagaa

SEQ ID NO: 447 - DNA, 14 bp, Artificial Sequence
  Synthetic Sequence
gctccgaccgctgg

SEQ ID NO: 448 - DNA, 18 bp, Artificial Sequence
  Synthetic Sequence
ctgggtgagaaaggcttc

SEQ ID NO: 449 - DNA, 17 bp, Artificial Sequence
  Synthetic Sequence
gcatgagaacctgggcc

SEQ ID NO: 450 - DNA, 18 bp, Artificial Sequence
  Synthetic Sequence
acttcgggatggcccgag

SEQ ID NO: 451 - DNA, 25 bp, Artificial Sequence
  Synthetic Sequence
cgaacaatgttctggtggttgaatt

SEQ ID NO: 452 - DNA, 15 bp, Artificial Sequence
  Synthetic Sequence
gcgcctttggggagg

SEQ ID NO: 453 - DNA, 17 bp, Artificial Sequence
  Synthetic Sequence
cacttcaggcagcgtct

SEQ ID NO: 454 - DNA, 24 bp, Artificial Sequence
  Synthetic Sequence
cacccaatcaagctcaacttcgta

SEQ ID NO: 455 - DNA, 17 bp, Artificial Sequence
  Synthetic Sequence
ccagaggcagaggtcga

SEQ ID NO: 456 - DNA, 21 bp, Artificial Sequence
  Synthetic Sequence
tgcctttaccactcagagaag

SEQ ID NO: 457 - DNA, 25 bp, Artificial Sequence
  Synthetic Sequence
tttaaaaagggttgaaaaagccgaa

SEQ ID NO: 458 - DNA, 30 bp, Artificial Sequence
  Synthetic Sequence
taccttatcaatgtctcgaatatttacatt

SEQ ID NO: 459 - DNA, 20 bp, Artificial Sequence
  Synthetic Sequence
cctgggattggaacaaggta

SEQ ID NO: 460 - DNA, 24 bp, Artificial Sequence
  Synthetic Sequence
ccaatagggttcagcaaatcttct

SEQ ID NO: 461 - DNA, 23 bp, Artificial Sequence
  Synthetic Sequence
tccatagaaaatctttctcctgc

SEQ ID NO: 462 - DNA, 23 bp, Artificial Sequence
  Synthetic Sequence
gagtcacacaccttttgtgtttc

SEQ ID NO: 463 - DNA, 30 bp, Artificial Sequence
  Synthetic Sequence
atttcatgaaacaaatgaatgatgcacatc

SEQ ID NO: 464 - DNA, 18 bp, Artificial Sequence
  Synthetic Sequence
cccccacagagcgctccc

SEQ ID NO: 465 - DNA, 17 bp, Artificial Sequence
  Synthetic Sequence
ggcgggcagtgtgtatg

SEQ ID NO: 466 - DNA, 17 bp, Artificial Sequence
  Synthetic Sequence
ccacagggatgccgggg

SEQ ID NO: 467 - DNA, 24 bp, Artificial Sequence
  Synthetic Sequence
gggccacatttgaacattgtaaac

SEQ ID NO: 468 - DNA, 19 bp, Artificial Sequence
  Synthetic Sequence
gcctggccagagacatcat

SEQ ID NO: 469 - DNA, 22 bp, Artificial Sequence
  Synthetic Sequence
tgggcaagacttctgcctattt

SEQ ID NO: 470 - DNA, 28 bp, Artificial Sequence
  Synthetic Sequence
ccttggtaatcacatgaatattgtgaat

SEQ ID NO: 471 - DNA, 19 bp, Artificial Sequence
  Synthetic Sequence
agacccaacacaacttcct

SEQ ID NO: 472 - DNA, 21 bp, Artificial Sequence
  Synthetic Sequence
attttggtctagccagagaca

SEQ ID NO: 473 - DNA, 18 bp, Artificial Sequence
  Synthetic Sequence
ggctccacttcccagcaa

SEQ ID NO: 474 - DNA, 18 bp, Artificial Sequence
  Synthetic Sequence
tgcccctctatgacctgc

SEQ ID NO: 475 - DNA, 17 bp, Artificial Sequence
  Synthetic Sequence
cagctttggtgccacct

SEQ ID NO: 476 - DNA, 15 bp, Artificial Sequence
  Synthetic Sequence
tgcccggcaggagtc

SEQ ID NO: 477 - DNA, 15 bp, Artificial Sequence
  Synthetic Sequence
cgcaccggagcccag

SEQ ID NO: 478 - DNA, 16 bp, Artificial Sequence
  Synthetic Sequence
gcatgagctgcgtgat

SEQ ID NO: 479 - DNA, 17 bp, Artificial Sequence
  Synthetic Sequence
ctggccaaactgctggg

SEQ ID NO: 480 - DNA, 30 bp, Artificial Sequence
  Synthetic Sequence
tctcagaacaataaactgaaatataccttc

SEQ ID NO: 481 - DNA, 17 bp, Artificial Sequence
  Synthetic Sequence
cagtgaagtggatggct

SEQ ID NO: 482 - DNA, 14 bp, Artificial Sequence
  Synthetic Sequence
atggtgcccgccga

SEQ ID NO: 483 - DNA, 22 bp, Artificial Sequence
  Synthetic Sequence
tcagcctggttgaagaagtcgt

SEQ ID NO: 484 - DNA, 25 bp, Artificial Sequence
  Synthetic Sequence
cctcacagtaaaaataggtgatttt

SEQ ID NO: 485 - DNA, 23 bp, Artificial Sequence
  Synthetic Sequence
gggacaaagaattggatctggat

SEQ ID NO: 486 - DNA, 23 bp, Artificial Sequence
  Synthetic Sequence
ttactctcgtctccacagacaca

SEQ ID NO: 487 - DNA, 17 bp, Artificial Sequence
  Synthetic Sequence
tggtggggactcgaact

SEQ ID NO: 488 - DNA, 20 bp, Artificial Sequence
  Synthetic Sequence
gagagctgcatcagttcact

SEQ ID NO: 489 - DNA, 25 bp, Artificial Sequence
  Synthetic Sequence
agacautaagaagauggccaagcaa

SEQ ID NO: 490 - DNA, 24 bp, Artificial Sequence
  Synthetic Sequence
attaatuggacacagugccagagt

SEQ ID NO: 491 - DNA, 24 bp, Artificial Sequence
  Synthetic Sequence
gcccattatucagagcgagtaugg

SEQ ID NO: 492 - DNA, 20 bp, Artificial Sequence
  Synthetic Sequence
gagcuggagcgcctgauaat

SEQ ID NO: 493 - DNA, 21 bp, Artificial Sequence
  Synthetic Sequence
ctatgttcutgtcgccuccga

SEQ ID NO: 494 - DNA, 22 bp, Artificial Sequence
  Synthetic Sequence
ggaagcucatugaagcagagga

SEQ ID NO: 495 - DNA, 19 bp, Artificial Sequence
  Synthetic Sequence
gctcaccaugtggttuggg

SEQ ID NO: 496 - DNA, 25 bp, Artificial Sequence
  Synthetic Sequence
agacattaagaagatggccaagcaa

SEQ ID NO: 497 - DNA, 24 bp, Artificial Sequence
  Synthetic Sequence
attaattggacacagtgccagagt

SEQ ID NO: 498 - DNA, 24 bp, Artificial Sequence
  Synthetic Sequence
gcccattattcagagcgagtatgg

SEQ ID NO: 499 - DNA, 20 bp, Artificial Sequence
  Synthetic Sequence
gagctggagcgcctgataat

SEQ ID NO: 500 - DNA, 21 bp, Artificial Sequence
  Synthetic Sequence
ctatgttcttgtcgcctccga

SEQ ID NO: 501 - DNA, 22 bp, Artificial Sequence
  Synthetic Sequence
ggaagctcattgaagcagagga

SEQ ID NO: 502 - DNA, 19 bp, Artificial Sequence
  Synthetic Sequence
gctcaccatgtggtttggg

SEQ ID NO: 503 - DNA, 21 bp, Artificial Sequence
  Synthetic Sequence
tggcccgcaucaauacaaact

SEQ ID NO: 504 - DNA, 19 bp, Artificial Sequence
  Synthetic Sequence
actgcccugtgctcacauc

SEQ ID NO: 505 - DNA, 25 bp, Artificial Sequence
  Synthetic Sequence
gatggtactgcuctagcagacttut

SEQ ID NO: 506 - DNA, 19 bp, Artificial Sequence
  Synthetic Sequence
cgaagcccucctgctcauc

SEQ ID NO: 507 - DNA, 23 bp, Artificial Sequence
  Synthetic Sequence
cctcuccaacacacaggaguaat

SEQ ID NO: 508 - DNA, 20 bp, Artificial Sequence
  Synthetic Sequence
gcugccacggatgtauacct

SEQ ID NO: 509 - DNA, 21 bp, Artificial Sequence
  Synthetic Sequence
tggcaaucgaatccagcucat

SEQ ID NO: 510 - DNA, 21 bp, Artificial Sequence
  Synthetic Sequence
tggcccgcatcaatacaaact

SEQ ID NO: 511 - DNA, 19 bp, Artificial Sequence
  Synthetic Sequence
actgccctgtgctcacatc

SEQ ID NO: 512 - DNA, 25 bp, Artificial Sequence
  Synthetic Sequence
gatggtactgctctagcagactttt

SEQ ID NO: 513 - DNA, 19 bp, Artificial Sequence
  Synthetic Sequence
cgaagccctcctgctcatc

SEQ ID NO: 514 - DNA, 23 bp, Artificial Sequence
  Synthetic Sequence
cctctccaacacacaggagtaat

SEQ ID NO: 515 - DNA, 20 bp, Artificial Sequence
  Synthetic Sequence
gctgccacggatgtatacct

SEQ ID NO: 516 - DNA, 21 bp, Artificial Sequence
  Synthetic Sequence
tggcaatcgaatccagctcat

SEQ ID NO: 517 - DNA, 18 bp, Artificial Sequence
  Synthetic Sequence
ccagctccctgcgaagag

SEQ ID NO: 518 - DNA, 28 bp, Artificial Sequence
  Synthetic Sequence
cctatcttggatgatggctggtgcaaag

SEQ ID NO: 519 - DNA, 20 bp, Artificial Sequence
  Synthetic Sequence
gacgggtccaactacacgtt

SEQ ID NO: 520 - DNA, 22 bp, Artificial Sequence
  Synthetic Sequence
cctggtgctccatgaggagaca

SEQ ID NO: 521 - DNA, 19 bp, Artificial Sequence
  Synthetic Sequence
gactcccatgacccccatc

SEQ ID NO: 522 - DNA, 21 bp, Artificial Sequence
  Synthetic Sequence
aggatgatggcactgaactcc

SEQ ID NO: 523 - DNA, 24 bp, Artificial Sequence
  Synthetic Sequence
cgtgtggtctgctcccttttcttg

SEQ ID NO: 524 - DNA, 20 bp, Artificial Sequence
  Synthetic Sequence
gcacattgctcccgttaagg

SEQ ID NO: 525 - DNA, 26 bp, Artificial Sequence
  Synthetic Sequence
gtgatccagactctgaccttttgcca

SEQ ID NO: 526 - DNA, 23 bp, Artificial Sequence
  Synthetic Sequence
acgaagtgcaatggtctttaggt

SEQ ID NO: 527 - DNA, 28 bp, Artificial Sequence
  Synthetic Sequence
caacttcagctatgaggtaatttttctc

SEQ ID NO: 528 - DNA, 28 bp, Artificial Sequence
  Synthetic Sequence
caacttcagctaugaggtaatttttcuc

SEQ ID NO: 529 - DNA, 22 bp, Artificial Sequence
  Synthetic Sequence
agaccaggagtcagactgtagg

SEQ ID NO: 530 - DNA, 22 bp, Artificial Sequence
  Synthetic Sequence
agaccaggagucagactguagg

SEQ ID NO: 531 - DNA, 22 bp, Artificial Sequence
  Synthetic Sequence
tcatcctcagggccatcttcat

SEQ ID NO: 532 - DNA, 22 bp, Artificial Sequence
  Synthetic Sequence
tcatccucagggccatctucat

SEQ ID NO: 533 - DNA, 18 bp, Artificial Sequence
  Synthetic Sequence
ccagctccctgcgaagag

SEQ ID NO: 534 - DNA, 18 bp, Artificial Sequence
  Synthetic Sequence
ccagcucccugcgaagag

SEQ ID NO: 535 - DNA, 20 bp, Artificial Sequence
  Synthetic Sequence
gtccttgttttgctgctggt

SEQ ID NO: 536 - DNA, 20 bp, Artificial Sequence
  Synthetic Sequence
gtccttgutttgctgcuggt

SEQ ID NO: 537 - DNA, 25 bp, Artificial Sequence
  Synthetic Sequence
cacttcagacgacacattccataca

SEQ ID NO: 538 - DNA, 25 bp, Artificial Sequence
  Synthetic Sequence
cactucagacgacacattccauaca

SEQ ID NO: 539 - DNA, 24 bp, Artificial Sequence
  Synthetic Sequence
cgtgtggtctgctcccttttcttg

SEQ ID NO: 540 - DNA, 24 bp, Artificial Sequence
  Synthetic Sequence
cgtgtggtcugctcccttttctug

SEQ ID NO: 541 - DNA, 19 bp, Artificial Sequence
  Synthetic Sequence
gcacagcggaactcactgg

SEQ ID NO: 542 - DNA, 19 bp, Artificial Sequence
  Synthetic Sequence
gcacagcggaacucacugg

SEQ ID NO: 543 - DNA, 19 bp, Artificial Sequence
  Synthetic Sequence
gaggcagcctccatgagtg

SEQ ID NO: 544 - DNA, 19 bp, Artificial Sequence
  Synthetic Sequence
gaggcagccuccatgagug

SEQ ID NO: 545 - DNA, 21 bp, Artificial Sequence
  Synthetic Sequence
atggtggatgtcgtgtagctt

SEQ ID NO: 546 - DNA, 21 bp, Artificial Sequence
  Synthetic Sequence
atggtggatgucgtgtagcut

SEQ ID NO: 547 - DNA, 26 bp, Artificial Sequence
  Synthetic Sequence
gtgatccagactctgaccttttgcca

SEQ ID NO: 548 - DNA, 26 bp, Artificial Sequence
  Synthetic Sequence
gtgatccagacuctgacctttugcca

SEQ ID NO: 549 - DNA, 23 bp, Artificial Sequence
  Synthetic Sequence
aagggtacatgagagccattacg

SEQ ID NO: 550 - DNA, 23 bp, Artificial Sequence
  Synthetic Sequence
aagggtacaugagagccatuacg

SEQ ID NO: 551 - DNA, 22 bp, Artificial Sequence
  Synthetic Sequence
gcggaagtgacattatcaacgc

SEQ ID NO: 552 - DNA, 22 bp, Artificial Sequence
  Synthetic Sequence
gcggaagugacattaucaacgc

SEQ ID NO: 553 - DNA, 19 bp, Artificial Sequence
  Synthetic Sequence
gactcccatgacccccatc

SEQ ID NO: 554 - DNA, 19 bp, Artificial Sequence
  Synthetic Sequence
gactcccaugacccccauc

SEQ ID NO: 555 - DNA, 24 bp, Artificial Sequence
  Synthetic Sequence
atcagagcttaaactgggaagctg

SEQ ID NO: 556 - DNA, 24 bp, Artificial Sequence
  Synthetic Sequence
atcagagctuaaactgggaagcug

SEQ ID NO: 557 - DNA, 22 bp, Artificial Sequence
  Synthetic Sequence
aagaatcttgtcccctgtggtg

SEQ ID NO: 558 - DNA, 22 bp, Artificial Sequence
  Synthetic Sequence
aagaatcttgucccctgtggug

SEQ ID NO: 559 - DNA, 20 bp, Artificial Sequence
  Synthetic Sequence
acgatcccgagactctgctt

SEQ ID NO: 560 - DNA, 20 bp, Artificial Sequence
  Synthetic Sequence
acgatcccgagacuctgcut

SEQ ID NO: 561 - DNA, 21 bp, Artificial Sequence
  Synthetic Sequence
aggatgatggcactgaactcc

SEQ ID NO: 562 - DNA, 21 bp, Artificial Sequence
  Synthetic Sequence
aggatgauggcactgaacucc

SEQ ID NO: 563 - DNA, 17 bp, Artificial Sequence
  Synthetic Sequence
ctgggtggcaccctctc

SEQ ID NO: 564 - DNA, 17 bp, Artificial Sequence
  Synthetic Sequence
ctggguggcaccctcuc

SEQ ID NO: 565 - DNA, 27 bp, Artificial Sequence
  Synthetic Sequence
actgcagacttaggaatcagtttactc

SEQ ID NO: 566 - DNA, 27 bp, Artificial Sequence
  Synthetic Sequence
actgcagactuaggaatcagtttacuc

SEQ ID NO: 567 - DNA, 28 bp, Artificial Sequence
  Synthetic Sequence
cctatcttggatgatggctggtgcaaag

SEQ ID NO: 568 - DNA, 28 bp, Artificial Sequence
  Synthetic Sequence
cctatcttggaugatggctggugcaaag

SEQ ID NO: 569 - DNA, 18 bp, Artificial Sequence
  Synthetic Sequence
ctgtgtgacggcagcgat

SEQ ID NO: 570 - DNA, 18 bp, Artificial Sequence
  Synthetic Sequence
cugtgugacggcagcgat

SEQ ID NO: 571 - DNA, 21 bp, Artificial Sequence
  Synthetic Sequence
ccagtcagtccagtagacctc

SEQ ID NO: 572 - DNA, 21 bp, Artificial Sequence
  Synthetic Sequence
ccagtcaguccagtagaccuc

SEQ ID NO: 573 - DNA, 22 bp, Artificial Sequence
  Synthetic Sequence
aatcgcatcttcttcagcgaca

SEQ ID NO: 574 - DNA, 22 bp, Artificial Sequence
  Synthetic Sequence
aatcgcaucttctucagcgaca

SEQ ID NO: 575 - DNA, 22 bp, Artificial Sequence
  Synthetic Sequence
cctggtgctccatgaggagaca

SEQ ID NO: 576 - DNA, 22 bp, Artificial Sequence
  Synthetic Sequence
cctggugctccaugaggagaca

SEQ ID NO: 577 - DNA, 29 bp, Artificial Sequence
  Synthetic Sequence
aaaatatgctagagttgtacagaagttgg

SEQ ID NO: 578 - DNA, 29 bp, Artificial Sequence
  Synthetic Sequence
aaaatatgctagagutgtacagaagtugg

SEQ ID NO: 579 - DNA, 19 bp, Artificial Sequence
  Synthetic Sequence
cgctggaactcgtctcact

SEQ ID NO: 580 - DNA, 19 bp, Artificial Sequence
  Synthetic Sequence
cgctggaacucgtcucact

SEQ ID NO: 581 - DNA, 23 bp, Artificial Sequence
  Synthetic Sequence
acgaagtgcaatggtctttaggt

SEQ ID NO: 582 - DNA, 23 bp, Artificial Sequence
  Synthetic Sequence
acgaagugcaatggtcttuaggt

SEQ ID NO: 583 - DNA, 28 bp, Artificial Sequence
  Synthetic Sequence
caacttcagctatgaggtaatttttctc

SEQ ID NO: 584 - DNA, 28 bp, Artificial Sequence
  Synthetic Sequence
caacttcagctaugaggtaatttttcuc

SEQ ID NO: 585 - DNA, 22 bp, Artificial Sequence
  Synthetic Sequence
tcatcctcagggccatcttcat

SEQ ID NO: 586 - DNA, 22 bp, Artificial Sequence
  Synthetic Sequence
tcatccucagggccatctucat

SEQ ID NO: 587 - DNA, 18 bp, Artificial Sequence
  Synthetic Sequence
ccagctccctgcgaagag

SEQ ID NO: 588 - DNA, 18 bp, Artificial Sequence
  Synthetic Sequence
ccagcucccugcgaagag

SEQ ID NO: 589 - DNA, 25 bp, Artificial Sequence
  Synthetic Sequence
cacttcagacgacacattccataca

SEQ ID NO: 590 - DNA, 25 bp, Artificial Sequence
  Synthetic Sequence
cactucagacgacacattccauaca

SEQ ID NO: 591 - DNA, 24 bp, Artificial Sequence
  Synthetic Sequence
cgtgtggtctgctcccttttcttg

SEQ ID NO: 592 - DNA, 24 bp, Artificial Sequence
  Synthetic Sequence
cgtgtggtcugctcccttttctug

SEQ ID NO: 593 - DNA, 24 bp, Artificial Sequence
  Synthetic Sequence
atcagagcttaaactgggaagctg

SEQ ID NO: 594 - DNA, 24 bp, Artificial Sequence
  Synthetic Sequence
atcagagctuaaactgggaagcug

SEQ ID NO: 595 - DNA, 20 bp, Artificial Sequence
  Synthetic Sequence
acgatcccgagactctgctt

SEQ ID NO: 596 - DNA, 20 bp, Artificial Sequence
  Synthetic Sequence
acgatcccgagacuctgcut

SEQ ID NO: 597 - DNA, 21 bp, Artificial Sequence
  Synthetic Sequence
aggatgatggcactgaactcc

SEQ ID NO: 598 - DNA, 21 bp, Artificial Sequence
  Synthetic Sequence
aggatgauggcactgaacucc

SEQ ID NO: 599 - DNA, 27 bp, Artificial Sequence
  Synthetic Sequence
actgcagacttaggaatcagtttactc

SEQ ID NO: 600 - DNA, 27 bp, Artificial Sequence
  Synthetic Sequence
actgcagactuaggaatcagtttacuc

SEQ ID NO: 601 - DNA, 28 bp, Artificial Sequence
  Synthetic Sequence
cctatcttggatgatggctggtgcaaag

SEQ ID NO: 602 - DNA, 28 bp, Artificial Sequence
  Synthetic Sequence
cctatcttggaugatggctggugcaaag